European Patent Specification EP 4 076 390 B1, published February 7, 2024. Title: Prebiotic and probiotic treatment to reduce oral dysbiosis and promote eubiosis. Applicant: Fundación para el Fomento de la Investigación Sanitaria y Biomédica de la Comunitat Valenciana. The sequence listing filed with the application follows.

SEQUENCE LISTING (11 sequences)

SEQ ID NO: 1 - RNA, 752 nt, Rothia dentocariosa
  D1P7 / CECT9999
taatcctgttcgctccccatgctttcgcttctcagcgtcagttacagcccagagacctgccttcgccatcggtgttcctcctgatatctgtgcattccaccgctacaccaggaattccagtctcccctactgcactctagttagcccgtacccactgcaaaaccggagttaagccccggcctttcacagcagacgcgaccaaccgcctacaagctctttacgcccaataattccggacaacgctcgcgccctacgtattaccgcggctgctggcacgtagttagccggcgctttctctgcacctaccgtcactttcgcttcttcgatgctaacagaggtttacaacccgaaggccgtcatccctcacgcggcgtcgctgcatcaggcttgcgcccattgtgcaatattccccactgctgcctcccgtaggagtctgggccgtgtctcagtcccagtgtggccggtcaccctctcaggccggctacccgtcgtcgccttggtaagccattacctcaccaacaagctgataggccgtgagcccatctaaaaccactccataacgctttccaccaacaccccatgcagagattggtcgtatccggtattagacccagtttcccaggcttatcccagagtcaaaggtaggtcactcacgtattactcacccgttcgccactaatccacggtgcaagcaccgcttcatcgttcgacttgcatgtgttaagcacgccgccagcgttcgtcctgagcct

SEQ ID NO: 2 - RNA, 752 nt, Rothia aeria
  D1P17 / CECT30000
ctaatcctgttcgctccccatgctttcgcttctcagcgtcagttacagcccagagacctgccttcgccatcggtgttcctcctgatatctgcgcattccaccgctacaccaggaattccagtctcccctactgcactctagttagcccgtacccactgcaaaaccagggttaagccccagcctttcacagcagacgcgaccaaccgcctacaagctctttacgcccaataattccggacaacgctcgcgccctacgtattaccgcggctgctggcacgtagttagccggcgctttctctgcacctaccgtcactttcgcttcttcgatgctaacagaggtttacaacccgaaggccgtcatccctcacgcggcgtcgctgcatcaggcttgcgcccattgtgcaatattccccactgctgcctcccgtaggagtctgggccgtgtctcagtcccagtgtggccggtcaccctctcaggccggctacccgtcgtcgccttggtaagccattacctcaccaacaagctgataggccgtgagcccatctaaaaccactccataacgctttccaccaacaccccatgcggagattggtcatatccggtattagacccagtttcccaggcttatcccagagtcaaaggtaggtcactcacgtattactcacccgttcgccactaatccacctagcaagctaggcttcatcgttcgacttgcatgtgttaagcacgccgccagcgttcgtcctgagca

SEQ ID NO: 3 - RNA, 752 nt, Rothia mucilaginosa
  D3T4 / CECT30001
taatcctgttcgctccccatgctttcgcttctcagcgtcagttacagcccagagacctgccttcgccatcggtgttcctcctgatatctgcgcattccaccgctacaccaggaattccagtctcccctactgcactctagtctgcccgtacccactgcaatacacggagttaagctccggcctttcacagcagacgcgacaaaccgcctacaagctctttacgcccaataattccggacaacgctcgcgccctacgtattaccgcggctgctggcacgtagttagccggcgctttctctgcaggtaccgtcaatctctcttcttccctgctaacagaggtttacaacccgaaggccgtcatccctcacgcggcgtcgctgcatcaggcttgcgcccattgtgcaatattccccactgctgcctcccgtaggagtctgggccgtgtctcagtcccagtgtggccggtcaccctctcaggccggctacccgtcgtcgccttggtgagccattacctcaccaacaagctgataggccgtgagcccatctataaccactacataacgctttccaccaacaccccatgcggagattggtcgtatccggtattagacccagtttcccaggcttatcccagagttaaaggtaggttactcacgtattactcacccgttcgccactaatccacctagcaagctaggcttcatcgttcgacttgcatgtgttaagcacgccgccagcgttcgtcctgagca

SEQ ID NO: 4 - RNA, 748 nt, Rothia mucilaginosa
  D4T4 / CECT30002
taatcctgttcgctccccatgctttcgcttctcagcgtcagttacagcccagagacctgccttcgccatcggtgttcctcctgatatctgcgcattccaccgctacaccaggaattccagtctcccctactgcactctagtctgcccgtacccactgcaatacacggagttaagctccggcctttcacagcagacgcgacaaaccgcctacaagctctttacgcccaataattccggacaacgctcgcgccctacgtattaccgcggctgctggcacgtagttagccggcgctttctctgcaggtaccgtcaatctctcttcttccctgctaacagaggtttacaacccgaaggccgtcatccctcacgcggcgtcgctgcatcaggcttgcgcccattgtgcaatattccccactgctgcctcccgtaggagtctgggccgtgtctcagtcccagtgtggccggtcaccctctcaggccggctacccgtcgtcgccttggtgagccgttacctcaccaacaagctgataggccgtgagcccatctataaccactacataacgctttccaccaacaccccatgcggagattggtcgtatccggtattagacccagtttcccaggcttatcccagagttaaaggtaggttactcacgtattactcacccgttcgccactaatccacctagcaagctaggcttcatcgttcgacttgcatgtgttaagcacgccgccagcgttcgtcctg

SEQ ID NO: 5 - RNA, 752 nt, Rothia mucilaginosa
  D4T6 / CECT30003
taatcctgttcgctccccatgctttcgcttctcagcgtcagttacagcccagagacctgccttcgccatcggtgttcctcctgatatctgcgcattccaccgctacaccaggaattccagtctcccctactgcactctagtctgcccgtacccactgcaatacacggagttaagctccggcctttcacagcagacgcgacaaaccgcctacaagctctttacgcccaataattccggacaacgctcgcgccctacgtattaccgcggctgctggcacgtagttagccggcgctttctctgcaggtaccgtcaatctctcttcttccctgctaacagaggtttacaacccgaaggccgtcatccctcacgcggcgtcgctgcatcaggcttgcgcccattgtgcaatattccccactgctgcctcccgtaggagtctgggccgtgtctcagtcccagtgtggccggtcaccctctcaggccggctacccgtcgtcgccttggtgagccgttacctcaccaacaagctgataggccgtgagcccatctataaccactacataacgctttccaccaacaccccatgcggagattggtcgtatccggtattagacccagtttcccaggcttatcccagagttaaaggtaggttactcacgtattactcacccgttcgccactaatccacctagcaagctaggcttcatcgttcgacttgcatgtgttaagcacgccgccagcgttcgtcctgagca

SEQ ID NO: 6 - RNA, 752 nt, Rothia mucilaginosa
  D4T9 / CECT30004
gtaatcctgttcgctccccatgctttcgcttctcagcgtcagttacagcccagagacctgccttcgccatcggtgttcctcctgatatctgcgcattccaccgctacaccaggaattccagtctcccctactgcactctagtctgcccgtacccactgcaatacacggagttaagctccggcctttcacagcagacgcgacaaaccgcctacaagctctttacgcccaataattccggacaacgctcgcgccctacgtattaccgcggctgctggcacgtagttagccggcgctttctctgcaggtaccgtcaatctctcttcttccctgctaacagaggtttacaacccgaaggccgtcatccctcacgcggcgtcgctgcatcaggcttgcgcccattgtgcaatattccccactgctgcctcccgtaggagtctgggccgtgtctcagtcccagtgtggccggtcaccctctcaggccggctacccgtcgtcgccttggtgagccgttacctcaccaacaagctgataggccgtgagcccatctataaccactacataacgctttccaccaacaccccatgcggagattggtcgtatccggtattagacccagtttcccaggcttatcccagagttaaaggtaggttactcacgtattactcacccgttcgccactaatccacctagcaagctaggcttcatcgttcgacttgcatgtgttaagcacgccgccagcgttcgtcctgagc

SEQ ID NO: 7 - RNA, 758 nt, Rothia mucilaginosa
  D5T11A / CECT30005
gagataatcctgttcgctccccatgctttcgcttctcagcgtcagttacagcccagagacctgccttcgccatcggtgttcctcctgatatctgcgcattccaccgctacaccaggaattccagtctcccctactgcactctagtctgcccgtacccactgcaatacacggagttaagccccggcctttcacagcagacgcgacaaaccgcctacaagctctttacgcccaataattccggacaacgctcgcgccctacgtattaccgcggctgctggcacgtagttagccggcgctttctctgcaggtaccgtcaatctctcttcttccctgctaacagaggtttacaacccgaaggccgtcatccctcacgcggcgtcgctgcatcaggcttgcgcccattgtgcaatattccccactgctgcctcccgtaggagtctgggccgtgtctcagtcccagtgtggccggtcaccctctcaggccggctacccgtcgtcgccttggtgagccgttacctcaccaacaagctgataggccgtgagcccatctataaccactacataacgctttccaccaacaccccatgcggagattggtcgtatccggtattagacccagtttcccgggcttatcccagagttaaaggtaggttactcacgtattactcacccgttcgccactaatccacctagcaagctaggcttcatcgttcgacttgcatgtgttaagcacgccgccagcgttcgtcctgagcaag

SEQ ID NO: 8 - DNA, 50 bp, Artificial Sequence
  Primer 16S Amplicon F for 16S rRNA determination
  misc_feature 42: /allele="W can be any nucleotide"
  misc_feature 46: /allele="W can be A or T"
tcgtcggcagcgtcagatgtgtataagagacagcctacgggnggcwgcag

SEQ ID NO: 9 - DNA, 55 bp, Artificial Sequence
  Primer 16S Amplicon R for 16S rRNA determination
  misc_feature 42: /allele="V: A or C or G"
gtctcgtgggctcggagatgtgtataagagacaggactachvgggtatctaatcc

SEQ ID NO: 10 - DNA, 20 bp, Artificial Sequence
  Primer 8-F
  misc_feature 12: /allele="M: A or C"
agagtttgatcmtggctcag

SEQ ID NO: 11 - DNA, 19 bp, Artificial Sequence
  Primer 785-R
ctaccagggtatctaatcc